European Patent Application EP 4 600 361 A1, published August 13, 2025. Title: DESIGN METHOD AND PRODUCTION METHOD FOR NUCLEIC ACID CONSTRUCT AND PROTEIN COMPLEX. Applicant: University of Tsukuba. Application EP 23874976.6, filed October 6, 2023. The sequence listing filed with the application follows.

SEQUENCE LISTING (94 sequences)

SEQ ID NO: 1 - protein, 14 aa, unidentified
LSFELLHAPATVCG

SEQ ID NO: 2 - protein, 14 aa, unidentified
VLSFELLHAPATVC

SEQ ID NO: 3 - protein, 14 aa, unidentified
FVFLVLLPLVSSQC

SEQ ID NO: 4 - protein, 14 aa, unidentified
MFVFLVLLPLVSSQ

SEQ ID NO: 5 - protein, 16 aa, unidentified
SGWTFGAGAALQIPFA

SEQ ID NO: 6 - protein, 16 aa, unidentified
GWTFGAGAALQIPFAM

SEQ ID NO: 7 - protein, 14 aa, unidentified
TRFQTLLALHRSYL

SEQ ID NO: 8 - protein, 16 aa, unidentified
RAAEIRASANLAATKM

SEQ ID NO: 9 - protein, 16 aa, unidentified
AAEIRASANLAATKMS

SEQ ID NO: 10 - protein, 16 aa, unidentified
GINITRFQTLLALHRS

SEQ ID NO: 11 - protein, 16 aa, unidentified
INITRFQTLLALHRSY

SEQ ID NO: 12 - protein, 14 aa, unidentified
QSLLIVNNATNVVI

SEQ ID NO: 13 - protein, 16 aa, unidentified
QSIIAYTMSLGAENSV

SEQ ID NO: 14 - protein, 15 aa, unidentified
QSIIAYTMSLGAENS

SEQ ID NO: 15 - protein, 14 aa, unidentified
GGFNFSQILPDPSK

SEQ ID NO: 16 - protein, 13 aa, unidentified
GGFNFSQILPDPS

SEQ ID NO: 17 - protein, 14 aa, unidentified
ESIVRFPNITNLCP

SEQ ID NO: 18 - protein, 14 aa, unidentified
PTESIVRFPNITNL

SEQ ID NO: 19 - protein, 16 aa, unidentified
RAAEIRASANLAATKM

SEQ ID NO: 20 - protein, 16 aa, unidentified
AAEIRASANLAATKMS

SEQ ID NO: 21 - protein, 16 aa, unidentified
GINITRFQTLLALHRS

SEQ ID NO: 22 - protein, 16 aa, unidentified
INITRFQTLLALHRSY

SEQ ID NO: 23 - protein, 14 aa, unidentified
QSLLIVNNATNVVI

SEQ ID NO: 24 - protein, 16 aa, unidentified
QSIIAYTMSLGAENSV

SEQ ID NO: 25 - protein, 15 aa, unidentified
QSIIAYTMSLGAENS

SEQ ID NO: 26 - protein, 15 aa, unidentified
ALNTLVKQLSSNFGA

SEQ ID NO: 27 - protein, 14 aa, unidentified
LNTLVKQLSSNFGA

SEQ ID NO: 28 - protein, 16 aa, unidentified
KTQSLLIVNNATNVVI

SEQ ID NO: 29 - protein, 14 aa, unidentified
LLIVNNATNVVIKV

SEQ ID NO: 30 - protein, 16 aa, unidentified
RAAEIRASANLAATKM

SEQ ID NO: 31 - protein, 15 aa, unidentified
AAEIRASANLAATKM

SEQ ID NO: 32 - protein, 14 aa, unidentified
SGWTFGAGAALQIP

SEQ ID NO: 33 - protein, 14 aa, unidentified
GWTFGAGAALQIPF

SEQ ID NO: 34 - protein, 14 aa, unidentified
NFNFNGLTGTGVLT

SEQ ID NO: 35 - protein, 14 aa, unidentified
CVNFNFNGLTGTGV

SEQ ID NO: 36 - protein, 14 aa, unidentified
ALNTLVKQLSSNFG

SEQ ID NO: 37 - protein, 15 aa, unidentified
QALNTLVKQLSSNFG

SEQ ID NO: 38 - protein, 14 aa, unidentified
TRFQTLLALHRSYL

SEQ ID NO: 39 - protein, 15 aa, unidentified
TRFQTLLALHRSYLT

SEQ ID NO: 40 - protein, 15 aa, unidentified
KTQSLLIVNNATNVV

SEQ ID NO: 41 - protein, 16 aa, unidentified
KTQSLLIVNNATNVVI

SEQ ID NO: 42 - protein, 14 aa, unidentified
DVVIGIVNNTVYDP

SEQ ID NO: 43 - protein, 14 aa, unidentified
CDVVIGIVNNTVYD

SEQ ID NO: 44 - protein, 14 aa, unidentified
EGVFVSNGTHWFVT

SEQ ID NO: 45 - protein, 14 aa, unidentified
RFQTLLALHRSYLT

SEQ ID NO: 46 - protein, 16 aa, unidentified
ITRFQTLLALHRSYLT

SEQ ID NO: 47 - protein, 14 aa, unidentified
LQIPFAMQMAYRFN

SEQ ID NO: 48 - protein, 15 aa, unidentified
LQIPFAMQMAYRFNG

SEQ ID NO: 49 - protein, 13 aa, unidentified
TESIVRFPNITNL

SEQ ID NO: 50 - protein, 14 aa, unidentified
TESIVRFPNITNLC

SEQ ID NO: 51 - protein, 14 aa, unidentified
SNLLLQYGSFCTQL

SEQ ID NO: 52 - protein, 15 aa, unidentified
CSNLLLQYGSFCTQL

SEQ ID NO: 53 - protein, 15 aa, unidentified
RFQTLLALHRSYLTP

SEQ ID NO: 54 - protein, 14 aa, unidentified
RFQTLLALHRSYLT

SEQ ID NO: 55 - protein, 14 aa, unidentified
TDEMIAQYTSALLA

SEQ ID NO: 56 - protein, 14 aa, unidentified
LYRLFRKSNLKPFE

SEQ ID NO: 57 - protein, 14 aa, unidentified
NYLYRLFRKSNLKP

SEQ ID NO: 58 - protein, 14 aa, unidentified
FVFLVLLPLVSSQC

SEQ ID NO: 59 - protein, 14 aa, unidentified
MFVFLVLLPLVSSQ

SEQ ID NO: 60 - protein, 14 aa, unidentified
ESIVRFPNITNLCP

SEQ ID NO: 61 - protein, 14 aa, unidentified
GNYNYLYRLFRKSN

SEQ ID NO: 62 - protein, 15 aa, unidentified
GNYNYLYRLFRKSNL

SEQ ID NO: 63 - protein, 14 aa, unidentified
MFVFLVLLPLVSSQ

SEQ ID NO: 64 - protein, 14 aa, unidentified
FVFLVLLPLVSSQC

SEQ ID NO: 65 - protein, 14 aa, unidentified
IPTNFTISVTTEIL

SEQ ID NO: 66 - protein, 13 aa, unidentified
PTNFTISVTTEIL

SEQ ID NO: 67 - protein, 14 aa, unidentified
INLVRDLPQGFSAL

SEQ ID NO: 68 - protein, 14 aa, unidentified
PINLVRDLPQGFSA

SEQ ID NO: 69 - protein, 15 aa, unidentified
VEAEVQIDRLITGRL

SEQ ID NO: 70 - protein, 16 aa, unidentified
KVEAEVQIDRLITGRL

SEQ ID NO: 71 - protein, 13 aa, unidentified
NTLVKQLSSNFGA

SEQ ID NO: 72 - protein, 14 aa, unidentified
LNTLVKQLSSNFGA

SEQ ID NO: 73 - protein, 14 aa, unidentified
QSLLIVNNATNVVI

SEQ ID NO: 74 - protein, 14 aa, unidentified
TQSLLIVNNATNVV

SEQ ID NO: 75 - protein, 14 aa, unidentified
DLFLPFFSNVTWFH

SEQ ID NO: 76 - protein, 13 aa, unidentified
TESIVRFPNITNL

SEQ ID NO: 77 - protein, 14 aa, unidentified
TESIVRFPNITNLC

SEQ ID NO: 78 - protein, 14 aa, unidentified
SNLLLQYGSFCTQL

SEQ ID NO: 79 - protein, 15 aa, unidentified
CSNLLLQYGSFCTQL

SEQ ID NO: 80 - protein, 15 aa, unidentified
RFQTLLALHRSYLTP

SEQ ID NO: 81 - protein, 14 aa, unidentified
RFQTLLALHRSYLT

SEQ ID NO: 82 - protein, 14 aa, unidentified
TDEMIAQYTSALLA

SEQ ID NO: 83 - protein, 17 aa, unidentified
FASVYAWNRKRIVTQQL

SEQ ID NO: 84 - protein, 14 aa, unidentified
YNYLYRLFRKSNLK

SEQ ID NO: 85 - protein, 18 aa, unidentified
QLIRAAEIRASANLAAGG

SEQ ID NO: 86 - DNA, 51 bp, unidentified
  source 1..51: mol_type = other DNA
ttcgcctctgtgtacgcctggaaccggaagcggatcgtgacccagcagctg

SEQ ID NO: 87 - DNA, 42 bp, unidentified
  source 1..42: mol_type = other DNA
tacaattacctgtaccggctgttccggaagtccaatctgaag

SEQ ID NO: 88 - DNA, 54 bp, unidentified
  source 1..54: mol_type = other DNA
cagctgatcagagccgccgagattagagcctctgccaatctggccgccggcggc

SEQ ID NO: 89 - DNA, 123 bp, unidentified
  source 1..123: mol_type = other DNA
atgagccccggcagagcctccagcgtgagcctgatgctgctgctgctgctgagcctggccgccaccgtgaaggccgccgccatcatcccccagtccagcgcctgccccaacaccgaggccaag

SEQ ID NO: 90 - DNA, 186 bp, unidentified
  source 1..186: mol_type = other DNA
gacttcctgcagaacgtgaaggtgaacctgaaggtgttcaacagcctgggcgccaaggtgtccagcagaagacccagcgactacctgaacagaagcaccagcccctggaccctgcacagaaacgaggaccccgacagataccccagcgtgatctgggaggcccagtgcagacaccagagatgcgtg

SEQ ID NO: 91 - DNA, 165 bp, unidentified
  source 1..165: mol_type = other DNA
aacgccgagggcaagctggaccaccacatgaacagcgtgctgatccagcaggagatcctggtgctgaagagagagcccgagagctgccccttcaccttcagagtggagaagatgctggtgggcgtgggctgcacctgcgtggccagcatcgtgagacaggccgcc

SEQ ID NO: 92 - DNA, 189 bp, unidentified
  source 1..189: mol_type = other DNA
atgctggactgcagagccgtgatcatgctgtggctgctgccctgggtgacccagggcctggccgtgcccagatccagcagccccgactgggcccagtgccagcagctgagcagaaacctgtgcatgctggcctggaacgcccacgcccccgccggccacatgaacctgctgagagaggaggaggacgag

SEQ ID NO: 93 - DNA, 195 bp, unidentified
  source 1..195: mol_type = other DNA
gagaccaagaacaacgtgcccagaatccagtgcgaggacggctgcgacccccagggcctgaaggacaacagccagttctgcctgcagagaatcagacagggcctggccttctacaagcacctgctggacagcgacatcttcaagggcgagcccgccctgctgcccgacagccccatggagcagctgcacaccagc

SEQ ID NO: 94 - DNA, 204 bp, unidentified
  source 1..204: mol_type = other DNA
ctgctgggcctgagccagctgctgcagcccgaggaccaccccagagagacccagcagatgcccagcctgtccagcagccagcagtggcagagacccctgctgagaagcaagatcctgagaagcctgcaggccttcctggccatcgccgccagagtgttcgcccacggcgccgccaccctgaccgagcccctggtgcccaccgcc